European Patent Application EP 4 445 911 A1, published October 16, 2024. Title: BISPECIFIC ANTIBODIES SPECIFICALLY BINDING TO KLEBSIELLA PNEUMONIAE O2 ANTIGEN AND O1 ANTIGEN AND COMPOSITIONS THEREOF. Applicant: Beijing Solobio Genetechnology Co., Ltd. The sequence listing filed with the application follows.

SEQUENCE LISTING (115 sequences)

SEQ ID NO: 1 - protein, 5 aa, synthetic construct
TYYWN

SEQ ID NO: 2 - protein, 16 aa, synthetic construct
NIHQSGTVYYNPSLKS

SEQ ID NO: 3 - protein, 16 aa, synthetic construct
NIHQSSTLYYNPSLKS

SEQ ID NO: 4 - protein, 16 aa, synthetic construct
NIHQSGTTYYNPSLKS

SEQ ID NO: 5 - protein, 13 aa, synthetic construct
ESDHGYKWNYFDY

SEQ ID NO: 6 - protein, 13 aa, synthetic construct
ESDDGYKWNYFDY

SEQ ID NO: 7 - protein, 13 aa, synthetic construct
ESDVGYKWNYFDY

SEQ ID NO: 8 - protein, 11 aa, synthetic construct
RASQTVTNYLA

SEQ ID NO: 9 - protein, 11 aa, synthetic construct
RASQIVTNYLA

SEQ ID NO: 10 - protein, 11 aa, synthetic construct
RASQVVTNYLA

SEQ ID NO: 11 - protein, 11 aa, synthetic construct
RASQVVTDYLA

SEQ ID NO: 12 - protein, 7 aa, synthetic construct
DMSIRAA

SEQ ID NO: 13 - protein, 7 aa, synthetic construct
DKSIRAA

SEQ ID NO: 14 - protein, 7 aa, synthetic construct
DMIIRAA

SEQ ID NO: 15 - protein, 10 aa, synthetic construct
QHRSNWPIFT

SEQ ID NO: 16 - protein, 10 aa, synthetic construct
QHRSNWPLFT

SEQ ID NO: 17 - protein, 121 aa, synthetic construct
QVQLQESGPGLVKPSETLSLTCTVSGGSLSTYYWNWIRQPPGKGLEWIANIHQSGTVYYNPSLKSRVTMSVDTSKNQFSLKLSSVTAADTAVYYCARESDHGYKWNYFDYWGQGTLVTVSS

SEQ ID NO: 18 - protein, 121 aa, synthetic construct
QVQLQESGPGLVKPSETLSLTCTVSGGAISTYYWNWIRQPPGKGLEWIANIHQSSTLYYNPSLKSRVTMSVDTSKNQFSLKLSSVTAADTAVYYCARESDDGYKWNYFDYWGQGTLVTVSS

SEQ ID NO: 19 - protein, 121 aa, synthetic construct
QVQLQESGPGLVKPSETLSLTCTVSGGSISTYYWNWIRQPPGKGLEWIANIHQSGTTYYNPSLKSRVTMSVDTSKNQFSLKLSSVTAADTAVYYCARESDDGYKWNYFDYWGQGTLVTVSS

SEQ ID NO: 20 - protein, 121 aa, synthetic construct
QVQLQESGPGLVKPSETLSLTCTVSGGSIDTYYWNWIRQPPGKGLEWIANIHQSGTVYYNPSLKSRVTMSVDTSKNQFSLKLSSVTAADTAVYYCARESDVGYKWNYFDYWGQGTLVTVSS

SEQ ID NO: 21 - protein, 108 aa, synthetic construct
EIVLTQSPATLSVSPGERATLSCRASQTVTNYLAWYQHKPGQAPRLLIFDMSIRAAGIPARFSGSGSGTEFTLTISSLQSEDFAVYYCQHRSNWPIFTFGQGTKVEIK

SEQ ID NO: 22 - protein, 108 aa, synthetic construct
EIVLTQSPASLSLSPGERATLSCRASQIVTNYLAWYQHKPGQAPRLLIFDMSIRAAGIPARFSGSGSGTDFTLTISSLEPEDFAVYYCQHRSNWPLFTFGPGTKVDIK

SEQ ID NO: 23 - protein, 108 aa, synthetic construct
EIVLTQSPATLSVSPGERATLSCRASQVVTNYLAWYQHKPGQAPRLLIFDKSIRAAGIPARFSGSGSGTEFTLTISSLQSEDFAVYYCQHRSNWPLFTFGQGTKVEIK

SEQ ID NO: 24 - protein, 108 aa, synthetic construct
EIVLTQSPATLSVSPGERATLSCRASQVVTDYLAWYQHKPGQAPRLLIFDMIIRAAGIPARFSGSGSGTEFTLTISSLQSEDFAVYYCQHRSNWPLFTFGQGTKVEIK

SEQ ID NO: 25 - protein, 108 aa, synthetic construct
EIVLTQSPATLSVSPGERATLSCRASQVVTNYLAWYQHKPGQAPRLLIFDMSIRAAGIPARFSGSGSGTEFTLTISSLQSEDFAVYYCQHRSNWPIFTFGQGTKVEIK

SEQ ID NO: 26 - protein, 121 aa, synthetic construct
QVQLQESGPGLVKPSETLSLTCTVSGGSLSTYYWNWIRQPPGKCLEWIANIHQSGTVYYNPSLKSRVTMSVDTSKNQFSLKLSSVTAADTAVYYCARESDHGYKWNYFDYWGQGTLVTVSS

SEQ ID NO: 27 - protein, 121 aa, synthetic construct
QVQLQESGPGLVKPSETLSLTCTVSGGAISTYYWNWIRQPPGKCLEWIANIHQSSTLYYNPSLKSRVTMSVDTSKNQFSLKLSSVTAADTAVYYCARESDDGYKWNYFDYWGQGTLVTVSS

SEQ ID NO: 28 - protein, 121 aa, synthetic construct
QVQLQESGPGLVKPSETLSLTCTVSGGSISTYYWNWIRQPPGKCLEWIANIHQSGTTYYNPSLKSRVTMSVDTSKNQFSLKLSSVTAADTAVYYCARESDDGYKWNYFDYWGQGTLVTVSS

SEQ ID NO: 29 - protein, 121 aa, synthetic construct
QVQLQESGPGLVKPSETLSLTCTVSGGSIDTYYWNWIRQPPGKCLEWIANIHQSGTVYYNPSLKSRVTMSVDTSKNQFSLKLSSVTAADTAVYYCARESDVGYKWNYFDYWGQGTLVTVSS

SEQ ID NO: 30 - protein, 108 aa, synthetic construct
EIVLTQSPATLSVSPGERATLSCRASQTVTNYLAWYQHKPGQAPRLLIFDMSIRAAGIPARFSGSGSGTEFTLTISSLQSEDFAVYYCQHRSNWPIFTFGCGTKVEIK

SEQ ID NO: 31 - protein, 108 aa, synthetic construct
EIVLTQSPASLSLSPGERATLSCRASQIVTNYLAWYQHKPGQAPRLLIFDMSIRAAGIPARFSGSGSGTDFTLTISSLEPEDFAVYYCQHRSNWPLFTFGCGTKVDIK

SEQ ID NO: 32 - protein, 108 aa, synthetic construct
EIVLTQSPATLSVSPGERATLSCRASQVVTNYLAWYQHKPGQAPRLLIFDKSIRAAGIPARFSGSGSGTEFTLTISSLQSEDFAVYYCQHRSNWPLFTFGCGTKVEIK

SEQ ID NO: 33 - protein, 108 aa, synthetic construct
EIVLTQSPATLSVSPGERATLSCRASQVVTDYLAWYQHKPGQAPRLLIFDMIIRAAGIPARFSGSGSGTEFTLTISSLQSEDFAVYYCQHRSNWPLFTFGCGTKVEIK

SEQ ID NO: 34 - protein, 108 aa, synthetic construct
EIVLTQSPATLSVSPGERATLSCRASQVVTNYLAWYQHKPGQAPRLLIFDMSIRAAGIPARFSGSGSGTEFTLTISSLQSEDFAVYYCQHRSNWPIFTFGCGTKVEIK

SEQ ID NO: 35 - protein, 5 aa, synthetic construct
NAWMY

SEQ ID NO: 36 - protein, 5 aa, synthetic construct
GYWMS

SEQ ID NO: 37 - protein, 19 aa, synthetic construct
RIRSYSDGGTTDYAALVEG

SEQ ID NO: 38 - protein, 17 aa, synthetic construct
NIKQDGSEQYYVDSVKG

SEQ ID NO: 39 - protein, 9 aa, synthetic construct
PSGDFYPAS

SEQ ID NO: 40 - protein, 16 aa, synthetic construct
DRGIKMGSVWYPSFDL

SEQ ID NO: 41 - protein, 16 aa, synthetic construct
RSSQNLLHSNGYNYLD

SEQ ID NO: 42 - protein, 11 aa, synthetic construct
RASRSISNYLN

SEQ ID NO: 43 - protein, 7 aa, synthetic construct
LSSNRAS

SEQ ID NO: 44 - protein, 7 aa, synthetic construct
AASTLQS

SEQ ID NO: 45 - protein, 9 aa, synthetic construct
MQALQTPYT

SEQ ID NO: 46 - protein, 9 aa, synthetic construct
QQSYSAPRT

SEQ ID NO: 47 - protein, 120 aa, synthetic construct
EVQLVESGGGLVRPGGSLRLSCVASGLTFSNAWMYWVRQAPGKGLEWLGRIRSYSDGGTTDYAALVEGRFTISRDDSINTVFLQMNNLKSEDTAVYYCGFPSGDFYPASWGQGTLVTVSS

SEQ ID NO: 48 - protein, 125 aa, synthetic construct
EVQLLESGGGLVQPGGSLRLSCAASGFIFSGYWMSWVRQAPGKGLEWVANIKQDGSEQYYVDSVKGRFTISRDNAKSSLYLQMNSLRTEDTAIFYCARDRGIKMGSVWYPSFDLWGQGTMVTVSS

SEQ ID NO: 49 - protein, 112 aa, synthetic construct
DIVMTQTPLSLPVSPGEPASISCRSSQNLLHSNGYNYLDWYVQKPGQSPQLLIYLSSNRASGVPDRFSGSGSGTDFTLKISRVEAEDVGVYYCMQALQTPYTFGQGTKLEIK

SEQ ID NO: 50 - protein, 107 aa, synthetic construct
EIVLTQSPSSLSASVGDRVTITCRASRSISNYLNWYQQKPGQPPKLLIYAASTLQSGVPSRFRGSGSGAHFTLIISSLQPEDFASYYCQQSYSAPRTFGGGTRLEIK

SEQ ID NO: 51 - protein, 120 aa, synthetic construct
EVQLVESGGGLVRPGGSLRLSCVASGLTFSNAWMYWVRQAPGKCLEWLGRIRSYSDGGTTDYAALVEGRFTISRDDSINTVFLQMNNLKSEDTAVYYCGFPSGDFYPASWGQGTLVTVSS

SEQ ID NO: 52 - protein, 125 aa, synthetic construct
EVQLLESGGGLVQPGGSLRLSCAASGFIFSGYWMSWVRQAPGKCLEWVANIKQDGSEQYYVDSVKGRFTISRDNAKSSLYLQMNSLRTEDTAIFYCARDRGIKMGSVWYPSFDLWGQGTMVTVSS

SEQ ID NO: 53 - protein, 112 aa, synthetic construct
DIVMTQTPLSLPVSPGEPASISCRSSQNLLHSNGYNYLDWYVQKPGQSPQLLIYLSSNRASGVPDRFSGSGSGTDFTLKISRVEAEDVGVYYCMQALQTPYTFGCGTKLEIK

SEQ ID NO: 54 - protein, 107 aa, synthetic construct
EIVLTQSPSSLSASVGDRVTITCRASRSISNYLNWYQQKPGQPPKLLIYAASTLQSGVPSRFRGSGSGAHFTLIISSLQPEDFASYYCQQSYSAPRTFGCGTRLEIK

SEQ ID NO: 55 - protein, 330 aa, synthetic construct
ASTKGPSVFPLAPSSKSTSGGTAALGCLVKDYFPEPVTVSWNSGALTSGVHTFPAVLQSSGLYSLSSVVTVPSSSLGTQTYICNVNHKPSNTKVDKKVEPKSCDKTHTCPPCPAPELLGGPSVFLFPPKPKDTLMISRTPEVTCVVVDVSHEDPEVKFNWYVDGVEVHNAKTKPREEQYNSTYRVVSVLTVLHQDWLNGKEYKCKVSNKALPAPIEKTISKAKGQPREPQVYTLPPSREEMTKNQVSLTCLVKGFYPSDIAVEWESNGQPENNYKTTPPVLDSDGSFFLYSKLTVDKSRWQQGNVFSCSVMHEALHNHYTQKSLSLSPGK

SEQ ID NO: 56 - protein, 327 aa, synthetic construct
ASTKGPSVFPLAPCSRSTSESTAALGCLVKDYFPEPVTVSWNSGALTSGVHTFPAVLQSSGLYSLSSVVTVPSSSLGTKTYTCNVDHKPSNTKVDKRVESKYGPPCPSCPAPEFLGGPSVFLFPPKPKDTLMISRTPEVTCVVVDVSQEDPEVQFNWYVDGVEVHNAKTKPREEQFNSTYRVVSVLTVLHQDWLNGKEYKCKVSNKGLPSSIEKTISKAKGQPREPQVYTLPPSQEEMTKNQVSLTCLVKGFYPSDIAVEWESNGQPENNYKTTPPVLDSDGSFFLYSRLTVDKSRWQEGNVFSCSVMHEALHNHYTQKSLSLSLGK

SEQ ID NO: 57 - protein, 107 aa, synthetic construct [sequence omitted]

SEQ ID NO: 58 - protein, 106 aa, synthetic construct
GQPKAAPSVTLFPPSSEELQANKATLVCLISDFYPGAVTVAWKADSSPVKAGVETTTPSKQSNNKYAASSYLSLTPEQWKSHRSYSCQVTHEGSTVEKTVAPTECS

SEQ ID NO: 59 - protein, 217 aa, synthetic construct
APELLGGPSVFLFPPKPKDTLMISRTPEVTCVVVDVSHEDPEVKFNWYVDGVEVHNAKTKPREEQYNSTYRVVSVLTVLHQDWLNGKEYKCKVSNKALPAPIEKTISKAKGQPREPQVYTLPPSREEMTKNQVSLTCLVKGFYPSDIAVEWESNGQPENNYKTTPPVLDSDGSFFLYSKLTVDKSRWQQGNVFSCSVMHEALHNHYTQKSLSLSPGK

SEQ ID NO: 60 - protein, 98 aa, synthetic construct
ASTKGPSVFPLAPSSKSTSGGTAALGCLVKDYFPEPVTVSWNSGALTSGVHTFPAVLQSSGLYSLSSVVTVPSSSLGTQTYICNVNHKPSNTKVDKKV

SEQ ID NO: 61 - protein, 354 aa, synthetic construct
EVQLLESGGGLVQPGGSLRLSCAASGFIFSGYWMSWVRQAPGKGLEWVANIKQDGSEQYYVDSVKGRFTISRDNAKSSLYLQMNSLRTEDTAIFYCARDRGIKMGSVWYPSFDLWGQGTMVTVSSGGGGSGGGGSQVQLQESGPGLVKPSETLSLTCTVSGGSIDTYYWNWIRQPPGKGLEWIANIHQSGTVYYNPSLKSRVTMSVDTSKNQFSLKLSSVTAADTAVYYCARESDVGYKWNYFDYWGQGTLVTVSSASTKGPSVFPLAPSSKSTSGGTAALGCLVKDYFPEPVTVSWNSGALTSGVHTFPAVLQSSGLYSLSSVVTVPSSSLGTQTYICNVNHKPSNTKVDKKV

SEQ ID NO: 62 - protein, 332 aa, synthetic construct
EIVLTQSPSSLSASVGDRVTITCRASRSISNYLNWYQQKPGQPPKLLIYAASTLQSGVPSRFRGSGSGAHFTLIISSLQPEDFASYYCQQSYSAPRTFGGGTRLEIKGGGGSGGGGSEIVLTQSPATLSVSPGERATLSCRASQVVTNYLAWYQHKPGQAPRLLIFDMSIRAAGIPARFSGSGSGTEFTLTISSLQSEDFAVYYCQHRSNWPIFTFGQGTKVEIKRTVAAPSVFIFPPSDEQLKSGTASVVCLLNNFYPREAKVQWKVDNALQSGNSQESVTEQDSKDSTYSLSSTLTLSKADYEKHKVYACEVTHQGLSSPVTKSFNRGEC

SEQ ID NO: 63 - protein, 349 aa, synthetic construct
EVQLVESGGGLVRPGGSLRLSCVASGLTFSNAWMYWVRQAPGKGLEWLGRIRSYSDGGTTDYAALVEGRFTISRDDSINTVFLQMNNLKSEDTAVYYCGFPSGDFYPASWGQGTLVTVSSGGGGSGGGGSQVQLQESGPGLVKPSETLSLTCTVSGGSIDTYYWNWIRQPPGKGLEWIANIHQSGTVYYNPSLKSRVTMSVDTSKNQFSLKLSSVTAADTAVYYCARESDVGYKWNYFDYWGQGTLVTVSSASTKGPSVFPLAPSSKSTSGGTAALGCLVKDYFPEPVTVSWNSGALTSGVHTFPAVLQSSGLYSLSSVVTVPSSSLGTQTYICNVNHKPSNTKVDKKV

SEQ ID NO: 64 - protein, 337 aa, synthetic construct
DIVMTQTPLSLPVSPGEPASISCRSSQNLLHSNGYNYLDWYVQKPGQSPQLLIYLSSNRASGVPDRFSGSGSGTDFTLKISRVEAEDVGVYYCMQALQTPYTFGQGTKLEIKGGGGSGGGGSEIVLTQSPATLSVSPGERATLSCRASQVVTNYLAWYQHKPGQAPRLLIFDMSIRAAGIPARFSGSGSGTEFTLTISSLQSEDFAVYYCQHRSNWPIFTFGQGTKVEIKRTVAAPSVFIFPPSDEQLKSGTASVVCLLNNFYPREAKVQWKVDNALQSGNSQESVTEQDSKDSTYSLSSTLTLSKADYEKHKVYACEVTHQGLSSPVTKSFNRGEC

SEQ ID NO: 65 - protein, 345 aa, synthetic construct
QVQLQESGPGLVKPSETLSLTCTVSGGSIDTYYWNWIRQPPGKGLEWIANIHQSGTVYYNPSLKSRVTMSVDTSKNQFSLKLSSVTAADTAVYYCARESDVGYKWNYFDYWGQGTLVTVSSASTKGPEVQLVESGGGLVRPGGSLRLSCVASGLTFSNAWMYWVRQAPGKGLEWLGRIRSYSDGGTTDYAALVEGRFTISRDDSINTVFLQMNNLKSEDTAVYYCGFPSGDFYPASWGQGTLVTVSSASTKGPSVFPLAPSSKSTSGGTAALGCLVKDYFPEPVTVSWNSGALTSGVHTFPAVLQSSGLYSLSSVVTVPSSSLGTQTYICNVNHKPSNTKVDKKV

SEQ ID NO: 66 - protein, 332 aa, synthetic construct
EIVLTQSPATLSVSPGERATLSCRASQVVTNYLAWYQHKPGQAPRLLIFDMSIRAAGIPARFSGSGSGTEFTLTISSLQSEDFAVYYCQHRSNWPIFTFGQGTKVEIKTVAAPDIVMTQTPLSLPVSPGEPASISCRSSQNLLHSNGYNYLDWYVQKPGQSPQLLIYLSSNRASGVPDRFSGSGSGTDFTLKISRVEAEDVGVYYCMQALQTPYTFGQGTKLEIKRTVAAPSVFIFPPSDEQLKSGTASVVCLLNNFYPREAKVQWKVDNALQSGNSQESVTEQDSKDSTYSLSSTLTLSKADYEKHKVYACEVTHQGLSSPVTKSFNRGEC

SEQ ID NO: 67 - protein, 350 aa, synthetic construct
QVQLQESGPGLVKPSETLSLTCTVSGGSIDTYYWNWIRQPPGKGLEWIANIHQSGTVYYNPSLKSRVTMSVDTSKNQFSLKLSSVTAADTAVYYCARESDVGYKWNYFDYWGQGTLVTVSSASTKGPEVQLLESGGGLVQPGGSLRLSCAASGFIFSGYWMSWVRQAPGKGLEWVANIKQDGSEQYYVDSVKGRFTISRDNAKSSLYLQMNSLRTEDTAIFYCARDRGIKMGSVWYPSFDLWGQGTMVTVSSASTKGPSVFPLAPSSKSTSGGTAALGCLVKDYFPEPVTVSWNSGALTSGVHTFPAVLQSSGLYSLSSVVTVPSSSLGTQTYICNVNHKPSNTKVDKKV

SEQ ID NO: 68 - protein, 327 aa, synthetic construct
EIVLTQSPATLSVSPGERATLSCRASQVVTNYLAWYQHKPGQAPRLLIFDMSIRAAGIPARFSGSGSGTEFTLTISSLQSEDFAVYYCQHRSNWPIFTFGQGTKVEIKTVAAPEIVLTQSPSSLSASVGDRVTITCRASRSISNYLNWYQQKPGQPPKLLIYAASTLQSGVPSRFRGSGSGAHFTLIISSLQPEDFASYYCQQSYSAPRTFGGGTRLEIKRTVAAPSVFIFPPSDEQLKSGTASVVCLLNNFYPREAKVQWKVDNALQSGNSQESVTEQDSKDSTYSLSSTLTLSKADYEKHKVYACEVTHQGLSSPVTKSFNRGEC

SEQ ID NO: 69 - protein, 487 aa, synthetic construct
EVQLLESGGGLVQPGGSLRLSCAASGFIFSGYWMSWVRQAPGKGLEWVANIKQDGSEQYYVDSVKGRFTISRDNAKSSLYLQMNSLRTEDTAIFYCARDRGIKMGSVWYPSFDLWGQGTMVTVSSASTKGPSVFPLAPSSKSTSGGTAALGCLVKDYFPEPVTVSWNSGALTSGVHTFPAVLQSSGLYSLSSVVTVPSSSLGTQTYICNVNHKPSNTKVDKKVEPKSCGGGGSGGGGSQVQLQESGPGLVKPSETLSLTCTVSGGSIDTYYWNWIRQPPGKCLEWIANIHQSGTVYYNPSLKSRVTMSVDTSKNQFSLKLSSVTAADTAVYYCARESDVGYKWNYFDYWGQGTLVTVSSGGGGSGGGGSGGGGSGGGGSEIVLTQSPATLSVSPGERATLSCRASQVVTNYLAWYQHKPGQAPRLLIFDMSIRAAGIPARFSGSGSGTEFTLTISSLQSEDFAVYYCQHRSNWPIFTFGCGTKVEIK

SEQ ID NO: 70 - protein, 214 aa, synthetic construct
EIVLTQSPSSLSASVGDRVTITCRASRSISNYLNWYQQKPGQPPKLLIYAASTLQSGVPSRFRGSGSGAHFTLIISSLQPEDFASYYCQQSYSAPRTFGGGTRLEIKRTVAAPSVFIFPPSDEQLKSGTASVVCLLNNFYPREAKVQWKVDNALQSGNSQESVTEQDSKDSTYSLSSTLTLSKADYEKHKVYACEVTHQGLSSPVTKSFNRGEC

SEQ ID NO: 71 - protein, 482 aa, synthetic construct
EVQLVESGGGLVRPGGSLRLSCVASGLTFSNAWMYWVRQAPGKGLEWLGRIRSYSDGGTTDYAALVEGRFTISRDDSINTVFLQMNNLKSEDTAVYYCGFPSGDFYPASWGQGTLVTVSSASTKGPSVFPLAPSSKSTSGGTAALGCLVKDYFPEPVTVSWNSGALTSGVHTFPAVLQSSGLYSLSSVVTVPSSSLGTQTYICNVNHKPSNTKVDKKVEPKSCGGGGSGGGGSQVQLQESGPGLVKPSETLSLTCTVSGGSIDTYYWNWIRQPPGKCLEWIANIHQSGTVYYNPSLKSRVTMSVDTSKNQFSLKLSSVTAADTAVYYCARESDVGYKWNYFDYWGQGTLVTVSSGGGGSGGGGSGGGGSGGGGSEIVLTQSPATLSVSPGERATLSCRASQVVTNYLAWYQHKPGQAPRLLIFDMSIRAAGIPARFSGSGSGTEFTLTISSLQSEDFAVYYCQHRSNWPIFTFGCGTKVEIK

SEQ ID NO: 72 - protein, 219 aa, synthetic construct
DIVMTQTPLSLPVSPGEPASISCRSSQNLLHSNGYNYLDWYVQKPGQSPQLLIYLSSNRASGVPDRFSGSGSGTDFTLKISRVEAEDVGVYYCMQALQTPYTFGQGTKLEIKRTVAAPSVFIFPPSDEQLKSGTASVVCLLNNFYPREAKVQWKVDNALQSGNSQESVTEQDSKDSTYSLSSTLTLSKADYEKHKVYACEVTHQGLSSPVTKSFNRGEC

SEQ ID NO: 73 - protein, 486 aa, synthetic construct
QVQLQESGPGLVKPSETLSLTCTVSGGSIDTYYWNWIRQPPGKGLEWIANIHQSGTVYYNPSLKSRVTMSVDTSKNQFSLKLSSVTAADTAVYYCARESDVGYKWNYFDYWGQGTLVTVSSASTKGPSVFPLAPSSKSTSGGTAALGCLVKDYFPEPVTVSWNSGALTSGVHTFPAVLQSSGLYSLSSVVTVPSSSLGTQTYICNVNHKPSNTKVDKKVEPKSCGGGGSGGGGSEVQLVESGGGLVRPGGSLRLSCVASGLTFSNAWMYWVRQAPGKGLEWLGRIRSYSDGGTTDYAALVEGRFTISRDDSINTVFLQMNNLKSEDTAVYYCGFPSGDFYPASWGQGTLVTVSSGGGGSGGGGSGGGGSGGGGSDIVMTQTPLSLPVSPGEPASISCRSSQNLLHSNGYNYLDWYVQKPGQSPQLLIYLSSNRASGVPDRFSGSGSGTDFTLKISRVEAEDVGVYYCMQALQTPYTFGQGTKLEIK

SEQ ID NO: 74 - protein, 215 aa, synthetic construct
EIVLTQSPATLSVSPGERATLSCRASQVVTNYLAWYQHKPGQAPRLLIFDMSIRAAGIPARFSGSGSGTEFTLTISSLQSEDFAVYYCQHRSNWPIFTFGQGTKVEIKRTVAAPSVFIFPPSDEQLKSGTASVVCLLNNFYPREAKVQWKVDNALQSGNSQESVTEQDSKDSTYSLSSTLTLSKADYEKHKVYACEVTHQGLSSPVTKSFNRGEC

SEQ ID NO: 75 - protein, 486 aa, synthetic construct
QVQLQESGPGLVKPSETLSLTCTVSGGSIDTYYWNWIRQPPGKGLEWIANIHQSGTVYYNPSLKSRVTMSVDTSKNQFSLKLSSVTAADTAVYYCARESDVGYKWNYFDYWGQGTLVTVSSASTKGPSVFPLAPSSKSTSGGTAALGCLVKDYFPEPVTVSWNSGALTSGVHTFPAVLQSSGLYSLSSVVTVPSSSLGTQTYICNVNHKPSNTKVDKKVEPKSCGGGGSGGGGSEVQLLESGGGLVQPGGSLRLSCAASGFIFSGYWMSWVRQAPGKGLEWVANIKQDGSEQYYVDSVKGRFTISRDNAKSSLYLQMNSLRTEDTAIFYCARDRGIKMGSVWYPSFDLWGQGTMVTVSSGGGGSGGGGSGGGGSGGGGSEIVLTQSPSSLSASVGDRVTITCRASRSISNYLNWYQQKPGQPPKLLIYAASTLQSGVPSRFRGSGSGAHFTLIISSLQPEDFASYYCQQSYSAPRTFGGGTRLEIK

SEQ ID NO: 76 - protein, 232 aa, synthetic construct
EVQLLESGGGLVQPGGSLRLSCAASGFIFSGYWMSWVRQAPGKGLEWVANIKQDGSEQYYVDSVKGRFTISRDNAKSSLYLQMNSLRTEDTAIFYCARDRGIKMGSVWYPSFDLWGQGTMVTVSSASVAAPSVFIFPPSDEQLKSGTASVVCLLNNFYPREAKVQWKVDNALQSGNSQESVTEQDSKDSTYSLSSTLTLSKADYEKHKVYACEVTHQGLSSPVTKSFNRGEC

SEQ ID NO: 77 - protein, 212 aa, synthetic construct
EIVLTQSPSSLSASVGDRVTITCRASRSISNYLNWYQQKPGQPPKLLIYAASTLQSGVPSRFRGSGSGAHFTLIISSLQPEDFASYYCQQSYSAPRTFGGGTRLEIKSSASTKGPSVFPLAPSSKSTSGGTAALGCLVKDYFPEPVTVSWNSGALTSGVHTFPAVLQSSGLYSLSSVVTVPSSSLGTQTYICNVNHKPSNTKVDKKVEPKSC

SEQ ID NO: 78 - protein, 219 aa, synthetic construct
QVQLQESGPGLVKPSETLSLTCTVSGGSIDTYYWNWIRQPPGKGLEWIANIHQSGTVYYNPSLKSRVTMSVDTSKNQFSLKLSSVTAADTAVYYCARESDVGYKWNYFDYWGQGTLVTVSSASTKGPSVFPLAPSSKSTSGGTAALGCLVKDYFPEPVTVSWNSGALTSGVHTFPAVLQSSGLYSLSSVVTVPSSSLGTQTYICNVNHKPSNTKVDKKV

SEQ ID NO: 79 - protein, 227 aa, synthetic construct
EVQLVESGGGLVRPGGSLRLSCVASGLTFSNAWMYWVRQAPGKGLEWLGRIRSYSDGGTTDYAALVEGRFTISRDDSINTVFLQMNNLKSEDTAVYYCGFPSGDFYPASWGQGTLVTVSSASVAAPSVFIFPPSDEQLKSGTASVVCLLNNFYPREAKVQWKVDNALQSGNSQESVTEQDSKDSTYSLSSTLTLSKADYEKHKVYACEVTHQGLSSPVTKSFNRGEC

SEQ ID NO: 80 - protein, 217 aa, synthetic construct
DIVMTQTPLSLPVSPGEPASISCRSSQNLLHSNGYNYLDWYVQKPGQSPQLLIYLSSNRASGVPDRFSGSGSGTDFTLKISRVEAEDVGVYYCMQALQTPYTFGQGTKLEIKSSASTKGPSVFPLAPSSKSTSGGTAALGCLVKDYFPEPVTVSWNSGALTSGVHTFPAVLQSSGLYSLSSVVTVPSSSLGTQTYICNVNHKPSNTKVDKKVEPKSC

SEQ ID NO: 81 - protein, 223 aa, synthetic construct
EVQLLESGGGLVQPGGSLRLSCAASGFIFSGYWMSWVRQAPGKGLEWVANIKQDGSEQYYVDSVKGRFTISRDNAKSSLYLQMNSLRTEDTAIFYCARDRGIKMGSVWYPSFDLWGQGTMVTVSSASTKGPSVFPLAPSSKSTSGGTAALGCLVKDYFPEPVTVSWNSGALTSGVHTFPAVLQSSGLYSLSSVVTVPSSSLGTQTYICNVNHKPSDTKVDKKV

SEQ ID NO: 82 - protein, 249 aa, synthetic construct
QVQLQESGPGLVKPSETLSLTCTVSGGSIDTYYWNWIRQPPGKGLEWIANIHQSGTVYYNPSLKSRVTMSVDTSKNQFSLKLSSVTAADTAVYYCARESDVGYKWNYFDYWGQGTLVTVSSGKPGSGKPGSGKPGSGKPGSEIVLTQSPATLSVSPGERATLSCRASQVVTNYLAWYQHKPGQAPRLLIFDMSIRAAGIPARFSGSGSGTEFTLTISSLQSEDFAVYYCQHRSNWPIFTFGQGTKVEIK

SEQ ID NO: 83 - protein, 214 aa, synthetic construct
EIVLTQSPSSLSASVGDRVTITCRASRSISNYLNWYQQKPGQPPKLLIYAASTLQSGVPSRFRGSGSGAHFTLIISSLQPEDFASYYCQQSYSAPRTFGGGTRLEIKRTVAAPSVFIFPPSDEQLKSGTASVVCLLNNFYPREAKVQWKVDNALQSGNSQESVTEQDSKDSTYSLSNTLTLSKADYEKHKVYACEVTHQGLSSPVTKSFNRGEC

SEQ ID NO: 84 - protein, 218 aa, synthetic construct
EVQLVESGGGLVRPGGSLRLSCVASGLTFSNAWMYWVRQAPGKGLEWLGRIRSYSDGGTTDYAALVEGRFTISRDDSINTVFLQMNNLKSEDTAVYYCGFPSGDFYPASWGQGTLVTVSSASTKGPSVFPLAPSSKSTSGGTAALGCLVKDYFPEPVTVSWNSGALTSGVHTFPAVLQSSGLYSLSSVVTVPSSSLGTQTYICNVNHKPSDTKVDKKV

SEQ ID NO: 85 - protein, 219 aa, synthetic construct
DIVMTQTPLSLPVSPGEPASISCRSSQNLLHSNGYNYLDWYVQKPGQSPQLLIYLSSNRASGVPDRFSGSGSGTDFTLKISRVEAEDVGVYYCMQALQTPYTFGQGTKLEIKRTVAAPSVFIFPPSDEQLKSGTASVVCLLNNFYPREAKVQWKVDNALQSGNSQESVTEQDSKDSTYSLSNTLTLSKADYEKHKVYACEVTHQGLSSPVTKSFNRGEC

SEQ ID NO: 86 - protein, 586 aa, synthetic construct
EVQLLESGGGLVQPGGSLRLSCAASGFIFSGYWMSWVRQAPGKGLEWVANIKQDGSEQYYVDSVKGRFTISRDNAKSSLYLQMNSLRTEDTAIFYCARDRGIKMGSVWYPSFDLWGQGTMVTVSSGGGGSGGGGSQVQLQESGPGLVKPSETLSLTCTVSGGSIDTYYWNWIRQPPGKGLEWIANIHQSGTVYYNPSLKSRVTMSVDTSKNQFSLKLSSVTAADTAVYYCARESDVGYKWNYFDYWGQGTLVTVSSASTKGPSVFPLAPSSKSTSGGTAALGCLVKDYFPEPVTVSWNSGALTSGVHTFPAVLQSSGLYSLSSVVTVPSSSLGTQTYICNVNHKPSNTKVDKKVEPKSCDKTHTCPPCPAPELLGGPSVFLFPPKPKDTLMISRTPEVTCVVVDVSHEDPEVKFNWYVDGVEVHNAKTKPREEQYNSTYRVVSVLTVLHQDWLNGKEYKCKVSNKALPAPIEKTISKAKGQPREPQVYTLPPSREEMTKNQVSLTCLVKGFYPSDIAVEWESNGQPENNYKTTPPVLDSDGSFFLYSKLTVDKSRWQQGNVFSCSVMHEALHNHYTQKSLSLSPGK

SEQ ID NO: 87 - protein, 581 aa, synthetic construct
EVQLVESGGGLVRPGGSLRLSCVASGLTFSNAWMYWVRQAPGKGLEWLGRIRSYSDGGTTDYAALVEGRFTISRDDSINTVFLQMNNLKSEDTAVYYCGFPSGDFYPASWGQGTLVTVSSGGGGSGGGGSQVQLQESGPGLVKPSETLSLTCTVSGGSIDTYYWNWIRQPPGKGLEWIANIHQSGTVYYNPSLKSRVTMSVDTSKNQFSLKLSSVTAADTAVYYCARESDVGYKWNYFDYWGQGTLVTVSSASTKGPSVFPLAPSSKSTSGGTAALGCLVKDYFPEPVTVSWNSGALTSGVHTFPAVLQSSGLYSLSSVVTVPSSSLGTQTYICNVNHKPSNTKVDKKVEPKSCDKTHTCPPCPAPELLGGPSVFLFPPKPKDTLMISRTPEVTCVVVDVSHEDPEVKFNWYVDGVEVHNAKTKPREEQYNSTYRVVSVLTVLHQDWLNGKEYKCKVSNKALPAPIEKTISKAKGQPREPQVYTLPPSREEMTKNQVSLTCLVKGFYPSDIAVEWESNGQPENNYKTTPPVLDSDGSFFLYSKLTVDKSRWQQGNVFSCSVMHEALHNHYTQKSLSLSPGK

SEQ ID NO: 88 - protein, 577 aa, synthetic construct
QVQLQESGPGLVKPSETLSLTCTVSGGSIDTYYWNWIRQPPGKGLEWIANIHQSGTVYYNPSLKSRVTMSVDTSKNQFSLKLSSVTAADTAVYYCARESDVGYKWNYFDYWGQGTLVTVSSASTKGPEVQLVESGGGLVRPGGSLRLSCVASGLTFSNAWMYWVRQAPGKGLEWLGRIRSYSDGGTTDYAALVEGRFTISRDDSINTVFLQMNNLKSEDTAVYYCGFPSGDFYPASWGQGTLVTVSSASTKGPSVFPLAPSSKSTSGGTAALGCLVKDYFPEPVTVSWNSGALTSGVHTFPAVLQSSGLYSLSSVVTVPSSSLGTQTYICNVNHKPSNTKVDKKVEPKSCDKTHTCPPCPAPELLGGPSVFLFPPKPKDTLMISRTPEVTCVVVDVSHEDPEVKFNWYVDGVEVHNAKTKPREEQYNSTYRVVSVLTVLHQDWLNGKEYKCKVSNKALPAPIEKTISKAKGQPREPQVYTLPPSREEMTKNQVSLTCLVKGFYPSDIAVEWESNGQPENNYKTTPPVLDSDGSFFLYSKLTVDKSRWQQGNVFSCSVMHEALHNHYTQKSLSLSPGK

SEQ ID NO: 89 - protein, 582 aa, synthetic construct
QVQLQESGPGLVKPSETLSLTCTVSGGSIDTYYWNWIRQPPGKGLEWIANIHQSGTVYYNPSLKSRVTMSVDTSKNQFSLKLSSVTAADTAVYYCARESDVGYKWNYFDYWGQGTLVTVSSASTKGPEVQLLESGGGLVQPGGSLRLSCAASGFIFSGYWMSWVRQAPGKGLEWVANIKQDGSEQYYVDSVKGRFTISRDNAKSSLYLQMNSLRTEDTAIFYCARDRGIKMGSVWYPSFDLWGQGTMVTVSSASTKGPSVFPLAPSSKSTSGGTAALGCLVKDYFPEPVTVSWNSGALTSGVHTFPAVLQSSGLYSLSSVVTVPSSSLGTQTYICNVNHKPSNTKVDKKVEPKSCDKTHTCPPCPAPELLGGPSVFLFPPKPKDTLMISRTPEVTCVVVDVSHEDPEVKFNWYVDGVEVHNAKTKPREEQYNSTYRVVSVLTVLHQDWLNGKEYKCKVSNKALPAPIEKTISKAKGQPREPQVYTLPPSREEMTKNQVSLTCLVKGFYPSDIAVEWESNGQPENNYKTTPPVLDSDGSFFLYSKLTVDKSRWQQGNVFSCSVMHEALHNHYTQKSLSLSPGK

SEQ ID NO: 90 - protein, 724 aa, synthetic construct
EVQLLESGGGLVQPGGSLRLSCAASGFIFSGYWMSWVRQAPGKGLEWVANIKQDGSEQYYVDSVKGRFTISRDNAKSSLYLQMNSLRTEDTAIFYCARDRGIKMGSVWYPSFDLWGQGTMVTVSSASTKGPSVFPLAPSSKSTSGGTAALGCLVKDYFPEPVTVSWNSGALTSGVHTFPAVLQSSGLYSLSSVVTVPSSSLGTQTYICNVNHKPSNTKVDKKVEPKSCGGGGSGGGGSQVQLQESGPGLVKPSETLSLTCTVSGGSIDTYYWNWIRQPPGKCLEWIANIHQSGTVYYNPSLKSRVTMSVDTSKNQFSLKLSSVTAADTAVYYCARESDVGYKWNYFDYWGQGTLVTVSSGGGGSGGGGSGGGGSGGGGSEIVLTQSPATLSVSPGERATLSCRASQVVTNYLAWYQHKPGQAPRLLIFDMSIRAAGIPARFSGSGSGTEFTLTISSLQSEDFAVYYCQHRSNWPIFTFGCGTKVEIKGGGGSGGGGSDKTHTCPPCPAPELLGGPSVFLFPPKPKDTLMISRTPEVTCVVVDVSHEDPEVKFNWYVDGVEVHNAKTKPREEQYNSTYRVVSVLTVLHQDWLNGKEYKCKVSNKALPAPIEKTISKAKGQPREPQVYTLPPSREEMTKNQVSLTCLVKGFYPSDIAVEWESNGQPENNYKTTPPVLDSDGSFFLYSKLTVDKSRWQQGNVFSCSVMHEALHNHYTQKSLSLSPGK

SEQ ID NO: 91 - protein, 719 aa, synthetic construct
EVQLVESGGGLVRPGGSLRLSCVASGLTFSNAWMYWVRQAPGKGLEWLGRIRSYSDGGTTDYAALVEGRFTISRDDSINTVFLQMNNLKSEDTAVYYCGFPSGDFYPASWGQGTLVTVSSASTKGPSVFPLAPSSKSTSGGTAALGCLVKDYFPEPVTVSWNSGALTSGVHTFPAVLQSSGLYSLSSVVTVPSSSLGTQTYICNVNHKPSNTKVDKKVEPKSCGGGGSGGGGSQVQLQESGPGLVKPSETLSLTCTVSGGSIDTYYWNWIRQPPGKCLEWIANIHQSGTVYYNPSLKSRVTMSVDTSKNQFSLKLSSVTAADTAVYYCARESDVGYKWNYFDYWGQGTLVTVSSGGGGSGGGGSGGGGSGGGGSEIVLTQSPATLSVSPGERATLSCRASQVVTNYLAWYQHKPGQAPRLLIFDMSIRAAGIPARFSGSGSGTEFTLTISSLQSEDFAVYYCQHRSNWPIFTFGCGTKVEIKGGGGSGGGGSDKTHTCPPCPAPELLGGPSVFLFPPKPKDTLMISRTPEVTCVVVDVSHEDPEVKFNWYVDGVEVHNAKTKPREEQYNSTYRVVSVLTVLHQDWLNGKEYKCKVSNKALPAPIEKTISKAKGQPREPQVYTLPPSREEMTKNQVSLTCLVKGFYPSDIAVEWESNGQPENNYKTTPPVLDSDGSFFLYSKLTVDKSRWQQGNVFSCSVMHEALHNHYTQKSLSLSPGK

SEQ ID NO: 92 - protein, 723 aa, synthetic construct
QVQLQESGPGLVKPSETLSLTCTVSGGSIDTYYWNWIRQPPGKGLEWIANIHQSGTVYYNPSLKSRVTMSVDTSKNQFSLKLSSVTAADTAVYYCARESDVGYKWNYFDYWGQGTLVTVSSASTKGPSVFPLAPSSKSTSGGTAALGCLVKDYFPEPVTVSWNSGALTSGVHTFPAVLQSSGLYSLSSVVTVPSSSLGTQTYICNVNHKPSNTKVDKKVEPKSCGGGGSGGGGSEVQLVESGGGLVRPGGSLRLSCVASGLTFSNAWMYWVRQAPGKGLEWLGRIRSYSDGGTTDYAALVEGRFTISRDDSINTVFLQMNNLKSEDTAVYYCGFPSGDFYPASWGQGTLVTVSSGGGGSGGGGSGGGGSGGGGSDIVMTQTPLSLPVSPGEPASISCRSSQNLLHSNGYNYLDWYVQKPGQSPQLLIYLSSNRASGVPDRFSGSGSGTDFTLKISRVEAEDVGVYYCMQALQTPYTFGQGTKLEIKGGGGSGGGGSDKTHTCPPCPAPELLGGPSVFLFPPKPKDTLMISRTPEVTCVVVDVSHEDPEVKFNWYVDGVEVHNAKTKPREEQYNSTYRVVSVLTVLHQDWLNGKEYKCKVSNKALPAPIEKTISKAKGQPREPQVYTLPPSREEMTKNQVSLTCLVKGFYPSDIAVEWESNGQPENNYKTTPPVLDSDGSFFLYSKLTVDKSRWQQGNVFSCSVMHEALHNHYTQKSLSLSPGK

SEQ ID NO: 93 - protein, 723 aa, synthetic construct
QVQLQESGPGLVKPSETLSLTCTVSGGSIDTYYWNWIRQPPGKGLEWIANIHQSGTVYYNPSLKSRVTMSVDTSKNQFSLKLSSVTAADTAVYYCARESDVGYKWNYFDYWGQGTLVTVSSASTKGPSVFPLAPSSKSTSGGTAALGCLVKDYFPEPVTVSWNSGALTSGVHTFPAVLQSSGLYSLSSVVTVPSSSLGTQTYICNVNHKPSNTKVDKKVEPKSCGGGGSGGGGSEVQLLESGGGLVQPGGSLRLSCAASGFIFSGYWMSWVRQAPGKGLEWVANIKQDGSEQYYVDSVKGRFTISRDNAKSSLYLQMNSLRTEDTAIFYCARDRGIKMGSVWYPSFDLWGQGTMVTVSSGGGGSGGGGSGGGGSGGGGSEIVLTQSPSSLSASVGDRVTITCRASRSISNYLNWYQQKPGQPPKLLIYAASTLQSGVPSRFRGSGSGAHFTLIISSLQPEDFASYYCQQSYSAPRTFGGGTRLEIKGGGGSGGGGSDKTHTCPPCPAPELLGGPSVFLFPPKPKDTLMISRTPEVTCVVVDVSHEDPEVKFNWYVDGVEVHNAKTKPREEQYNSTYRVVSVLTVLHQDWLNGKEYKCKVSNKALPAPIEKTISKAKGQPREPQVYTLPPSREEMTKNQVSLTCLVKGFYPSDIAVEWESNGQPENNYKTTPPVLDSDGSFFLYSKLTVDKSRWQQGNVFSCSVMHEALHNHYTQKSLSLSPGK

SEQ ID NO: 94 - protein, 459 aa, synthetic construct
EVQLLESGGGLVQPGGSLRLSCAASGFIFSGYWMSWVRQAPGKGLEWVANIKQDGSEQYYVDSVKGRFTISRDNAKSSLYLQMNSLRTEDTAIFYCARDRGIKMGSVWYPSFDLWGQGTMVTVSSASVAAPSVFIFPPSDEQLKSGTASVVCLLNNFYPREAKVQWKVDNALQSGNSQESVTEQDSKDSTYSLSSTLTLSKADYEKHKVYACEVTHQGLSSPVTKSFNRGECDKTHTCPPCPAPELLGGPSVFLFPPKPKDTLMISRTPEVTCVVVDVSHEDPEVKFNWYVDGVEVHNAKTKPREEQYNSTYRVVSVLTVLHQDWLNGKEYKCKVSNKALPAPIEKTISKAKGQPREPQVCTLPPSRDELTKNQVSLSCAVKGFYPSDIAVEWESNGQPENNYKTTPPVLDSDGSFFLVSKLTVDKSRWQQGNVFSCSVMHEALHNHYTQKSLSLSPGK

SEQ ID NO: 95 - protein, 451 aa, synthetic construct
QVQLQESGPGLVKPSETLSLTCTVSGGSIDTYYWNWIRQPPGKGLEWIANIHQSGTVYYNPSLKSRVTMSVDTSKNQFSLKLSSVTAADTAVYYCARESDVGYKWNYFDYWGQGTLVTVSSASTKGPSVFPLAPSSKSTSGGTAALGCLVKDYFPEPVTVSWNSGALTSGVHTFPAVLQSSGLYSLSSVVTVPSSSLGTQTYICNVNHKPSNTKVDKKVEPKSCDKTHTCPPCPAPELLGGPSVFLFPPKPKDTLMISRTPEVTCVVVDVSHEDPEVKFNWYVDGVEVHNAKTKPREEQYNSTYRVVSVLTVLHQDWLNGKEYKCKVSNKALPAPIEKTISKAKGQPREPQVYTLPPCRDELTKNQVSLWCLVKGFYPSDIAVEWESNGQPENNYKTTPPVLDSDGSFFLYSKLTVDKSRWQQGNVFSCSVMHEALHNHYTQKSLSLSPGK

SEQ ID NO: 96 - protein, 454 aa, synthetic construct
EVQLVESGGGLVRPGGSLRLSCVASGLTFSNAWMYWVRQAPGKGLEWLGRIRSYSDGGTTDYAALVEGRFTISRDDSINTVFLQMNNLKSEDTAVYYCGFPSGDFYPASWGQGTLVTVSSASVAAPSVFIFPPSDEQLKSGTASVVCLLNNFYPREAKVQWKVDNALQSGNSQESVTEQDSKDSTYSLSSTLTLSKADYEKHKVYACEVTHQGLSSPVTKSFNRGECDKTHTCPPCPAPELLGGPSVFLFPPKPKDTLMISRTPEVTCVVVDVSHEDPEVKFNWYVDGVEVHNAKTKPREEQYNSTYRVVSVLTVLHQDWLNGKEYKCKVSNKALPAPIEKTISKAKGQPREPQVCTLPPSRDELTKNQVSLSCAVKGFYPSDIAVEWESNGQPENNYKTTPPVLDSDGSFFLVSKLTVDKSRWQQGNVFSCSVMHEALHNHYTQKSLSLSPGK

SEQ ID NO: 97 - protein, 717 aa, synthetic construct
EVQLLESGGGLVQPGGSLRLSCAASGFIFSGYWMSWVRQAPGKGLEWVANIKQDGSEQYYVDSVKGRFTISRDNAKSSLYLQMNSLRTEDTAIFYCARDRGIKMGSVWYPSFDLWGQGTMVTVSSASTKGPSVFPLAPSSKSTSGGTAALGCLVKDYFPEPVTVSWNSGALTSGVHTFPAVLQSSGLYSLSSVVTVPSSSLGTQTYICNVNHKPSNTKVDKKVEPKSCDKTHTCPPCPAPELLGGPSVFLFPPKPKDTLMISRTPEVTCVVVDVSHEDPEVKFNWYVDGVEVHNAKTKPREEQYNSTYRVVSVLTVLHQDWLNGKEYKCKVSNKALPAPIEKTISKAKGQPREPQVYTLPPSRDELTKNQVSLTCLVKGFYPSDIAVEWESNGQPENNYKTTPPVLDSDGSFFLYSKLTVDKSRWQQGNVFSCSVMHEALHNHYTQKSLSLSPGGGGSGGGGTGGGGSQVQLQESGPGLVKPSETLSLTCTVSGGSIDTYYWNWIRQPPGKGLEWIANIHQSGTVYYNPSLKSRVTMSVDTSKNQFSLKLSSVTAADTAVYYCARESDVGYKWNYFDYWGQGTLVTVSSGGGGSGGGGSGGGGSGGGGSEIVLTQSPATLSVSPGERATLSCRASQVVTNYLAWYQHKPGQAPRLLIFDMSIRAAGIPARFSGSGSGTEFTLTISSLQSEDFAVYYCQHRSNWPIFTFGQGTKVEIK

SEQ ID NO: 98 - protein, 712 aa, synthetic construct
EVQLVESGGGLVRPGGSLRLSCVASGLTFSNAWMYWVRQAPGKGLEWLGRIRSYSDGGTTDYAALVEGRFTISRDDSINTVFLQMNNLKSEDTAVYYCGFPSGDFYPASWGQGTLVTVSSASTKGPSVFPLAPSSKSTSGGTAALGCLVKDYFPEPVTVSWNSGALTSGVHTFPAVLQSSGLYSLSSVVTVPSSSLGTQTYICNVNHKPSNTKVDKKVEPKSCDKTHTCPPCPAPELLGGPSVFLFPPKPKDTLMISRTPEVTCVVVDVSHEDPEVKFNWYVDGVEVHNAKTKPREEQYNSTYRVVSVLTVLHQDWLNGKEYKCKVSNKALPAPIEKTISKAKGQPREPQVYTLPPSRDELTKNQVSLTCLVKGFYPSDIAVEWESNGQPENNYKTTPPVLDSDGSFFLYSKLTVDKSRWQQGNVFSCSVMHEALHNHYTQKSLSLSPGGGGSGGGGTGGGGSQVQLQESGPGLVKPSETLSLTCTVSGGSIDTYYWNWIRQPPGKGLEWIANIHQSGTVYYNPSLKSRVTMSVDTSKNQFSLKLSSVTAADTAVYYCARESDVGYKWNYFDYWGQGTLVTVSSGGGGSGGGGSGGGGSGGGGSEIVLTQSPATLSVSPGERATLSCRASQVVTNYLAWYQHKPGQAPRLLIFDMSIRAAGIPARFSGSGSGTEFTLTISSLQSEDFAVYYCQHRSNWPIFTFGQGTKVEIK

SEQ ID NO: 99 - protein, 455 aa, synthetic construct
EVQLLESGGGLVQPGGSLRLSCAASGFIFSGYWMSWVRQAPGKGLEWVANIKQDGSEQYYVDSVKGRFTISRDNAKSSLYLQMNSLRTEDTAIFYCARDRGIKMGSVWYPSFDLWGQGTMVTVSSASTKGPSVFPLAPSSKSTSGGTAALGCLVKDYFPEPVTVSWNSGALTSGVHTFPAVLQSSGLYSLSSVVTVPSSSLGTQTYICNVNHKPSDTKVDKKVEPKSCDKTHTCPPCPAPELLGGPSVFLFPPKPKDTLMISRTPEVTCVVVDVSHEDPEVKFNWYVDGVEVHNAKTKPREEEYNSTYRVVSVLTVLHQDWLNGKEYKCKVSNKALPAPIEKTISKAKGQPREPQVYTLPPSREEMTKNQVSLTCDVSGFYPSDIAVEWESDGQPENNYKTTPPVLDSDGSFFLYSKLTVDKSRWEQGDVFSCSVMHEALHNHYTQKSLSLSPGK

SEQ ID NO: 100 - protein, 481 aa, synthetic construct
QVQLQESGPGLVKPSETLSLTCTVSGGSIDTYYWNWIRQPPGKGLEWIANIHQSGTVYYNPSLKSRVTMSVDTSKNQFSLKLSSVTAADTAVYYCARESDVGYKWNYFDYWGQGTLVTVSSGKPGSGKPGSGKPGSGKPGSEIVLTQSPATLSVSPGERATLSCRASQVVTNYLAWYQHKPGQAPRLLIFDMSIRAAGIPARFSGSGSGTEFTLTISSLQSEDFAVYYCQHRSNWPIFTFGQGTKVEIKEPKSSDKTHTCPPCPAPELLGGPSVFLFPPKPKDTLMISRTPEVTCVVVDVSHEDPEVKFNWYVDGVEVHNAKTKPREEQYNSTYRVVSVLTVLHQDWLNGKEYKCKVSNKALPAPIEKTISKAKGQPREPQVYTLPPSREQMTKNQVKLTCLVKGFYPSDIAVEWESNGQPENNYKTTPPVLDSDGSFFLYSKLTVDKSRWQQGNVFSCSVMHEALHNHYTQKSLSLSPGK

SEQ ID NO: 101 - protein, 450 aa, synthetic construct
EVQLVESGGGLVRPGGSLRLSCVASGLTFSNAWMYWVRQAPGKGLEWLGRIRSYSDGGTTDYAALVEGRFTISRDDSINTVFLQMNNLKSEDTAVYYCGFPSGDFYPASWGQGTLVTVSSASTKGPSVFPLAPSSKSTSGGTAALGCLVKDYFPEPVTVSWNSGALTSGVHTFPAVLQSSGLYSLSSVVTVPSSSLGTQTYICNVNHKPSDTKVDKKVEPKSCDKTHTCPPCPAPELLGGPSVFLFPPKPKDTLMISRTPEVTCVVVDVSHEDPEVKFNWYVDGVEVHNAKTKPREEEYNSTYRVVSVLTVLHQDWLNGKEYKCKVSNKALPAPIEKTISKAKGQPREPQVYTLPPSREEMTKNQVSLTCDVSGFYPSDIAVEWESDGQPENNYKTTPPVLDSDGSFFLYSKLTVDKSRWEQGDVFSCSVMHEALHNHYTQKSLSLSPGK

SEQ ID NO: 102 - protein, 10 aa, synthetic construct
GGGGSGGGGS

SEQ ID NO: 103 - protein, 20 aa, synthetic construct
GGGGSGGGGSGGGGSGGGGS

SEQ ID NO: 104 - protein, 15 aa, synthetic construct
GGGGSGGGGSGGGGS

SEQ ID NO: 105 - protein, 6 aa, synthetic construct
ASTKGP

SEQ ID NO: 106 - protein, 5 aa, synthetic construct
TVAAP

SEQ ID NO: 107 - protein, 17 aa, synthetic construct
EPKSDKTGGGGSGGGGS

SEQ ID NO: 108 - protein, 18 aa, synthetic construct
EPKSCGKTGGGGSGGGGS

SEQ ID NO: 109 - protein, 15 aa, synthetic construct
EPKSCGGGGSGGGGS

SEQ ID NO: 110 - protein, 24 aa, synthetic construct
GGGGSGGGGSEPKSDKTHTCPPCP

SEQ ID NO: 111 - protein, 15 aa, synthetic construct
GGGGSGGGGSCPPCP

SEQ ID NO: 112 - protein, 20 aa, synthetic construct
GGGGSGGGGSDKTHTCPPCP

SEQ ID NO: 113 - protein, 20 aa, synthetic construct
GKPGSGKPGSGKPGSGKPGS

SEQ ID NO: 114 - protein, 15 aa, synthetic construct
GGGGSGGGGTGGGGS

SEQ ID NO: 115 - protein, 577 aa, synthetic construct
QVQLQESGPGLVKPSETLSLTCTVSGGSIDTYYWNWIRQPPGKGLEWIANIHQSGTVYYNPSLKSRVTMSVDTSKNQFSLKLSSVTAADTAVYYCARESDVGYKWNYFDYWGQGTLVTVSSASTKGPEVQLVESGGGLVRPGGSLRLSCVASGLTFSNAWMYWVRQAPGKGLEWLGRIRSYSDGGTTDYAALVEGRFTISRDDSINTVFLQMNNLKSEDTAVYYCGFPSGDFYPASWGQGTLVTVSSASTKGPSVFPLAPSSKSTSGGTAALGCLVKDYFPEPVTVSWNSGALTSGVHTFPAVLQSSGLYSLSSVVTVPSSSLGTQTYICNVNHKPSNTKVDKKVEPKSCDKTHTCPPCPAPELLGGPSVFLFPPKPKDTLMISRTPEVTCVVVDVSHEDPEVKFNWYVDGVEVHNAKTKPREEQYNSTYRVVSVLTVLHQDWLNGKEYKCKVSNKALPAPIEKTISKAKGQPREPQVYTLPPSREEMTKNQVSLTCLVKGFYPSDIAVEWESNGQPENNYKTTPPVLDSDGSFFLYSKLTVDKSRWQQGNVFSCSVLHEALHSHYTQKSLSLSPGK